European Patent Application EP 4 641 189 A1, published October 29, 2025. Title: An enzyme electrode and an enzyme sensor. Applicant: Kikkoman Corporation. Application JP. The sequence listing filed with the application follows.

SEQUENCE LISTING (2 sequences)

SEQ ID NO: 1 - protein, 500 aa, Pichia kudriavzevii
MGSDSPRSISVDEFVKHNSQNDCWIAINGKVYDFTDFIPNHPGGVPPLVNHCGYDGTKLYEKLHPKGTIEKFLPKDKFLGVLDGEAPKLEADYLVDDDEQERLDYLNNLPPLSSIQNVYDFEYLAKKILPKDAWAYYSCGADDEITMRENHYAFQRVYFRPRICVDVKEVDTSYEMLGTKTSVPFYVSATALAKLGHPDGECSIARGAGKEGVVQMISTLSSMSLDEIAAARIPGATQWFQLYINEDRNVAKGLVKHAEDLGMKAIFITVDAPSLGNREKDKRLKFVNDTDVDLGDSADRNSGASKALSSFIDASVSWNDVKAVKSWTKLPVLVKGVQTVEDVIEAFDAGCQGVVLSNHGGRQLDTAPPPIELLAETVPTLKRLGKLRPDFEILIDGGVKRGTDILKAVAIGGQDVRVSVGMGRPLLYANSCYGEAGVRKLIQNLKDELEMDMRLLGVTKMDQLSSKHVDTKRLIGRDAINYLYDNVYSPIETVKFNNED

SEQ ID NO: 2 - DNA, 1503 bp, Pichia kudriavzevii
  source 1..1503: mol_type = other DNA
atggggtcagatagtcctagaagcattagcgttgacgaattcgttaaacacaacagccagaatgattgttggattgccattaatggaaaagtttatgatttcacggatttcattcctaaccacccagggggtgtcccacccctggtgaatcactgcggttacgacggtacgaaactgtatgaaaaactgcatcctaaaggtaccattgaaaaatttttaccgaaagataaatttcttggcgtgttagacggcgaggctccgaagctggaggcggattacctggttgacgacgacgaacaggaaagactggactacttgaacaatttgccgcctttatccagtattcagaatgtctacgacttcgagtatttggcaaaaaagattctgcctaaggatgcttgggcctactacagctgcggtgcagatgacgagataacgatgcgcgaaaaccattatgcgtttcaacgcgtttacttccgtccgcgcatttgcgttgatgtgaaggaagttgatactagctatgaaatgctgggtactaaaaccagcgtgccgttttatgttagtgccaccgcattggcgaaactgggtcatcccgatggtgagtgctcaattgcacgtggcgctggtaaggaaggtgtcgttcagatgatttcaactctgtcatcaatgagtctggatgaaatagcggcggcacggattccaggggcgacccagtggtttcagctgtatattaatgaggatcgtaatgtcgctaagggtctggttaaacatgcagaagacctgggtatgaaggcaatttttataaccgtggacgcaccgtccttaggcaatcgtgagaaggataagcgtctgaaatttgttaacgacacggatgtagatctgggggactcagccgaccgtaattcgggagcgtccaaggctctgagttcgtttatagatgcaagtgtttcttggaacgatgtgaaagccgtgaagtcgtggaccaaattacccgtgctggttaaaggagttcagaccgtggaagatgtaatagaagcctttgatgcaggttgtcagggggtcgtactgtctaaccatggagggcgccaactggacactgccccaccaccgatcgaacttctggcagagacggtgccgacattgaaacgtttaggcaaattacgcccggattttgaaatcttaatcgatggcggcgtgaaacgtgggacagacatattaaaagccgtggcgatcggcggccaagatgtaagagtatctgtaggcatgggacgcccattattatatgctaactcttgttatggagaggcgggagtccggaaattgatccaaaatttgaaagatgagcttgaaatggatatgcgccttcttggcgtcacaaaaatggatcaactttcttctaaacatgtagatacaaaacggcttatcggacgggatgctatcaactatctttatgataatgtatattcccctatcgaaacagtcaaatttaataatgaagattaa